European Patent Specification EP 3 765 506 B1, published April 24, 2024. Title: ANTI-CD25 ANTIBODY AGENTS. Applicant: TUSK THERAPEUTICS LTD CANCER RESEARCH TECHNOLOGY LIMITED. The sequence listing filed with the application follows.

SEQUENCE LISTING (10 sequences)

SEQ ID NO: 1 - protein, 119 aa, homo sapiens
QVQLQESGPGLVKPSETLSLTCTVSGFSLTSYGIQWIRQPPGKGLEWIGVIWAGGSTNYNSALMSRVTISKDNSKNQFSLKLSSVTAADTAVYYCARAYGYDGSWLAYWGQGTLVTVSS

SEQ ID NO: 2 - protein, 119 aa, homo sapiens
QVQLQESGPGLVKPSETLSLTCTVSGFSLTSYGIQWVRQPPGKGLEWIGVIWAGGSTNYNSALMSRVTISKDNSKSQFSLKLSSVTAADTAVYYCARAYGYDGSWLAYWGQGTLVTVSS

SEQ ID NO: 3 - protein, 119 aa, homo sapiens
QVQLVESGGGVVQPGGSLRLSCAVSGFSLTSYGIQWVRQAPGKGLEWVSVIWAGGSTNYNSALMSRFTISKDNSKSTLYLQMNSLRAEDTAVYYCARAYGYDGSWLAYWGQGTLVTVSS

SEQ ID NO: 4 - protein, 106 aa, homo sapiens
EIVLTQSPATLSLSPGERATLSCRASSSVSYMHWYQQKPGQAPRPLIFATSNLASGIPARFSGSGSGTDFTLTISSLEPEDFAVYYCQQWSSNPPTFGGGTKLEIK

SEQ ID NO: 5 - protein, 106 aa, homo sapiens
QIVLTQSPATLSLSPGERATLSCRASSSVSYMHWYQQKPGQAPRPLIFATSNLASGIPARFSGSGSGTDYTLTISSLEPEDFAVYYCQQWSSNPPTFGGGTKLEIK

SEQ ID NO: 6 - protein, 106 aa, homo sapiens
DIQMTQSPSSLSASVGDRVTITCRASSSVSYMHWYQQKPGKAPKPLIFATSNLASGVPSRFSGSGSGTDYTLTISSLQPEDFATYYCQQWSSNPPTFGGGTKLEIK

SEQ ID NO: 7 - protein, 106 aa, homo sapiens
QIQLTQSPSSLSASVGDRVTITCRASSSVSYMHWYQQKPGKSPKPLIFATSNLASGVPSRFSGSGSGTDYTLTISSLQPEDFATYYCQQWSSNPPTFGGGTKLEIK

SEQ ID NO: 8 - protein, 272 aa, homo sapiens
MDSYLLMWGLLTFIMVPGCQAELCDDDPPEIPHATFKAMAYKEGTMLNCECKRGFRRIKSGSLYMLCTGNSSHSSWDNQCQCTSSATRNTTKQVTPQPEEQKERKTTEMQSPMQPVDQASLPGHCREPPPWENEATERIYHFVVGQMVYYQCVQGYRALHRGPAESVCKMTHGKTRWTQPQLICTGEMETSQFPGEEKPQASPEGRPESETSCLVTTTDFQIQTEMAATMETSIFTTEYQVAVAGCVFLLISVLLLSGLTWQRRQRKSRRTI

SEQ ID NO: 9 - protein, 14 aa, Homo sapiens
YQCVQGYRALHRGP

SEQ ID NO: 10 - protein, 15 aa, Homo sapiens
SVCKMTHGKTRWTQP